European Patent Specification EP 4 013 497 B1, published October 4, 2023. Title: COMPOUNDS SUITABLE FOR THE TREATMENT AND PROPHYLAXIS OF MUSCLE WASTING AND OTHER CONDITIONS. Applicant: Adams, Volker Labeit, Siegfried. The sequence listing filed with the application follows.

SEQUENCE LISTING (6 sequences)

SEQ ID NO: 1 - DNA, 25 bp, Artificial Sequence
  PCR Primer
ctcatggactgattatggacaggac

SEQ ID NO: 2 - DNA, 25 bp, Artificial Sequence
  PCR Primer
gcaggtcagcaaagaacttatagcc

SEQ ID NO: 3 - DNA, 19 bp, Artificial Sequence
  PCR Primer
gatgtgcaaggaacacgaa

SEQ ID NO: 4 - DNA, 20 bp, Artificial Sequence
  PCR Primer
ccttcacctggtggctattc

SEQ ID NO: 5 - DNA, 26 bp, Artificial Sequence
  PCR Primer
gcacaaggagcaagtaggcacctcac

SEQ ID NO: 6 - DNA, 22 bp, Artificial Sequence
  PCR Primer
gcctggtgagccccaaacacct